European Patent Application EP 4 574 997 A1, published June 25, 2025. Title: Reduced PDE4D7 expression in prostate cancer correlates with down-regulation of genomic elements within the up-stream PDE4D coding region on chromosome 5 and provides prognostic information. Applicant: Koninklijke Philips N.V. Application EP. The sequence listing filed with the application follows.

SEQUENCE LISTING (8 sequences)

SEQ ID NO: 1 - DNA, 391 bp, Homo sapiens
  source 1..391: mol_type = genomic DNA
aatgtcattcccaaagtttactccatcgcacctggccactctgcccttgaccctcgactcagccaaatatgacatatctctggaaggctggcagatgcaagctgaacggttggccataagagcccagctgaaacaagagtacctgcttcagtacaacaaccaactctaaccaccaagggctcatcgaagatcttgccttaattcgttggacctatgcaagatcagcaaatgtctattctaatttcagactcactcctaaaactcactcttgggagctctgtgtggaattgggcccctcttcttctggtattatgttttcaaaactgacagggataggaaagaaaaacttatccaggaaggaaaattggatggaacatttaacatctcatat

SEQ ID NO: 2 - DNA, 98 bp, Homo sapiens
  source 1..98: mol_type = genomic DNA
atctgtgctctttgattacagttgttcaaccagttactaatctaactaattgtaactggttgaacaactgaacccaaagggtgcaaagtagaaacatt

SEQ ID NO: 3 - DNA, 339 bp, Homo sapiens
  source 1..339: mol_type = genomic DNA
agtcagtattttgacttaaattatatcaaatctacagatcagttgatggaccactgcaatttttatgatttggagacttctgatccagggacatgttcttttagggaaggatgtagagcaaaagatatgcataaacttgtgaaactttaccactgttcagaattcctcagagagagaaactacattcatcttggaaatccatattgcgtactttgaagaactgcagttcttcttgcaaactctttatttctttgaagttaggtcaggagaataatacggcatcattctgtggacaagccatggttattgccaccaaataaaatgtctctgtatcaagaa

SEQ ID NO: 4 - DNA, 465 bp, Homo sapiens
  source 1..465: mol_type = genomic DNA
gctgcaagtggcaccaagtcactcaatgacatgcaacaagaacaactggacacagctttatacctcctgagagcagtgttaggagaaagcaggagcagaccctgtctttaatgtcctggtggtggaccatttcaagtccatcctcaagaagcacatcttagcaacagggatatcaatgaagttcttgagagcatcccagctctctctctgtctaagatgtcacatccctcattacatctcaatgtccctctcagcctgcgctcccaggctccagatacagctgcgaagcctctattacaaacatattcctttgccgatgctgacccctcattgttatttgttttagacccagattggcaagttcccccaaaataaacaagtcagtattttgacttaaattatatcaaatctacagatcagttgatggaccactgcaatttttatgatttggagacttctgatcca

SEQ ID NO: 5 - DNA, 105 bp, Homo sapiens
  source 1..105: mol_type = genomic DNA
gtttgctttggcagaacatatactaaacttggaacaacacagagaagattagcatgaccctcacacaaggattacatgcaagttcctgaagcgttccatattttc

SEQ ID NO: 6 - DNA, 217 bp, Homo sapiens
  source 1..217: mol_type = genomic DNA
aaacagcctccttcaaaatgcagcttgactgtgattcatggcacaaagctggaataaccctgccagttcttagaagctttaagattcatcgtcttgaacttgatacacatagtatagcaccttaaaaacgaatcatctgctagttcagtattttctacttacaatcactccctcccagggcatgtaattaatttactgagcttaaaaaaaaaatatc

SEQ ID NO: 7 - DNA, 892 bp, Homo sapiens
  source 1..892: mol_type = genomic DNA
atggcccccaaatgccagtctccactcctgcctcaaaagaagaaaccaagaatgcctcctgctctgggaccggaggagacattggcctctgcaggcttgctgaggaagggagaaaaagaacagcaagaagcaattgaatgcattgatgaagtacaaaatgaaatagacagacttaatgaagaagccagtgaggagattttgaaagtagaacagaaatatgacaaactctgccaaccattttttcagaagatgtcagaattgatcgccaaaatcccaaattttggggtaacaacatttgtcaagcatccacaagtgtctgccctgctggaggaggatgaagaggcactgcattatttgagcagagttgaaatgacagaatttgaagatattaaatcaggttacagaatagatttttattttgatgaaaatctttactttgaaaataaacttctatccaaagaatttcatctgaatgagagtggtgatccatcttcaaagtccactgaaatgaaatggaaatctggaaaggatttgatgaaatgttcatctggaaaggatttgatgaaatgttcaagtcaaatgcagaataaagccagcaggaagaggcagcatgaggaaccagagagcttctttacctggtttactgaccattctgatgcaggtgctgatgagttatgagaggtcaccaaagatgatatttggtcaaactcattacagtactacttggttcccgatatggatgatgaagaagcagaatgagaagaagatgatgatgatgatgaagaggaggaaggataaaaagatactaatgaagaagacaatgaagatgaaggtgaagatgaagatgatgatgaaggggaggaaggagagaaggatgaaggaaaagattact

SEQ ID NO: 8 - DNA, 3240 bp, Homo sapiens
  source 1..3240: mol_type = genomic DNA
aatcacttagctcctcataacaagtctaactggctctggaaagctgaaagggctgcactggaacaacacagatgagatattctacacattaatctacttatctggaatcactttgcctctaaaggccagagaaaaatcacagcttccttgtcggaggggaaaaggacaggtgatctggggaaaacgcagctacacctggagcaaggtctcttcccggcttggcaatctcagctgtgccggcgctacgggacccgagccgtcccagaaaccaaagggcaggcacggcagcaaacgcctgagcctgccttgtacttcatgcaggttgaacagaaatgttttctgagcatgtattgttacagccctctgagatggtataaaagaatgaaagaagacacgacctgccttccaggagtttcacaaaaaagatgggatgaacacagtgttcacttccaccttccaccctttcactatgaaggaccctcaccagatggtggcaccatgctctcggacttcccagcctccagaactggacgggtaaattgaagcaaaaagcagacaagttctatgggatttgctggcattgatttcccaggatggcaaagtgctaagaactaaacctttaaagctaacaaaatgtactgatgtctttgcaaagtatccaagaccaacaagaaagtaatttcccacctcaccctaccaccacccagaaaaggagcacagagatggggaagagagtggctgcatctggcatccagccagaggagtccgtgcagggattctggatccctcttcccccaccccactgcccttccccctccaccccagcgttttggagaagcaagaaactgtgatgatgcagctccctcaagtatcacatgaagatagtggaaagagcctcctgaggtaaatatgccatgtagacagaaacaagcaatggctcaacagcaatgtatgaggtccaaggaccaggaccaaagggaaaaacagccatctcaccagacacctgcctacgaccagatgcgtcatctccaatattagctaactccctggaacctggactcaaggtgtgaaataaaggttaatgggaaaccgcaggagtcaaaaggagggggcaggattattgaggattcaggctgttgagaaatgaaagtttggatcactccccagataaagaaccttgaccatttaagggcaatggaaatacagaataggcagtagaagaaggaagccatagataccaactatggcctctcaatcaattacaaaactgagaattctgacagttttgtgtatttcctctttgcatgtgatgtatatgtgtgtatttgtatatattaaccattttcctttttctctcttcattattttatgaaagttgttgaatataaactctacaatttagcctttaggtaagagaatattcagtgggactttgatttgaggagtatttaagacagccagatgagactacgataactgttggaactgtgtgtctcctcatttggggaaaggggtgagaactctgcatttctctgaagaacagagttgactttgtgttatacagagttcaaatatatatataaaatggtgcatgtggaagctaagaagccaaaggagttcaccaagacagttatcaatatattgcctctccgctccaaatccacccttctttgccctgttccacgatactaatctggctcctcggtcagccagtgcaatgtcatctgttgctggtagagtgtaggggagacactacaaggtatagtaaaggggtcagatgcggtgtctcatgcctgtaatcacagccctttgggaggcagaggcaggaggatcacctgaggccaggagtttgagaccagcctggacaacatggtaaaaccccatctctactgaaaatacaaaattagcacgcacctgtaatcccagctactcgggaggctgaggcaggagaatcacttgaacctgggaggtggaggttgcagtgagccaagatcgcatcattgcactccagccagggaaaaaaggcaaaactctgtctcaaaaaaataaataaataaaataaaataaaacaaggtatagcaaataaaggagcattccttcttgattcttcctggttcttgttacctgtggccgccaccagtggtgtatgggagagtcaccctacagtgagttccaccagcacctagtgagggcttcctactgagttttattgtcacccgagcaggcaatttccttgccagcagtatgcaggagacccaatggtgaccaccttccagtgggtttttccagcaccctagaaggcacttttttgaccacagtgctgatccactggcacccaacagccagtaccctactcaccaggcctggcctgtggcacctcaaagaacttttctatcctgcgggccacagcaccaccctctccaacaaggtctgaatctcagccttcaggtgtgaaagacccttccatgtttgttcttttcttgggtatcctccctcagtcctagaagtagcagctcttccctatgtttgctatttctgtgttatttagcatacaatttaccccttttgtagtttatcacattttgccagttaataattctttatagtaaatgttccctcttcaaattactatctctcaccaaacactgacttctatatcctcatcagacactgagtgacacaacctccttcagaaaagaatccctttcaccctgcccttcatgatgaacactctcaacaaattaggtatagcaggaacataccttgacataataaaggccatatatgacgagcccacagctaacatcatactgaatggggaataactgaaagcctttcctctaagaactagaataagacaaggacacctactctaagcactcttattcggcattatactggaagtcctagccagactttctctttccggaaagagaaagaaatgaaaggcatccaaactggaaaacaggatgccagccagttgtggtggctcaagcctgtaatcccagcacttcgggaggctgaggtgggcagattgcttgaacccaggagttcaaatccagactagacaacatgatgaaaccctgtctctatgaaaaatacaaaaattagccaggtgtggtggcacacacctgtagtcccaactactcaggaggctgaggtgggaggatcacttgagcctgggaaatagaggatgcagtgagtcaagatcacaccagagcactccagcctggatgacag